European Patent Application EP 4 116 437 A1, published January 11, 2023. Title: A METHOD OF SCREENING FOR COLORECTAL CANCER. Applicant: Clinical Genomics Pty. Ltd. The sequence listing filed with the application follows.

SEQUENCE LISTING (76 sequences)

SEQ ID NO: 1 - DNA, 102 bp, homo sapiens
cagtgcccgaggcggcggcgagtacacgtggcgggctggattgcagaccggccctctcgcggcggagactcgcgacctagcggattgcatcagcaggaagac

SEQ ID NO: 2 - DNA, 87 bp, homo sapiens
agatcccaagggtcgtagcccctggccgtgtggaccgggtctgcggctgcagagcgcggtcccggctgcagcaagacctggggcagt

SEQ ID NO: 3 - DNA, 95 bp, homo sapiens
gacgacgcaccctctccgtgtcccgctctgcgcccttctgcgcgccccgctccctgtaccggagcagcgatccgggaggcggccgagaggtgcgc

SEQ ID NO: 4 - DNA, 92 bp, homo sapiens
ccggagttgcggctgagacgcgcgccgcgcgagccgggggactcggcgacggggcggggacgggacgacgcaccctctccgtgtcccgctct

SEQ ID NO: 5 - DNA, 110 bp, homo sapiens
cgcctgccctccgcgctcctgcgacggggtcgccacaagctggacgggatgagctaaccggactgtcggggccccaggagtggctgaggcggggccgtccaaggcaccca

SEQ ID NO: 6 - DNA, 299 bp, homo sapiens
caggaagctgcagcagaaggaggaggcggcggccaccccggaccccgccgcccggactcccgactcggaagtcgcgcccgccgctccggtcccgaccccgggaccccctgccgcagccgccacccctgggcccccagcggacgagctgtacgcggcgctggaggactatcaccctgccgagctgtaccgcgcgctcgccgtgtccgggggcaccctgccccgccgaaaggtgcgtcccccgcccgccttcaggatctgctcagcccctctccgactccctacagggcctgctgactccg

SEQ ID NO: 7 - DNA, 258 bp, homo sapiens
gacagagacagccccaggcaagttgaaggtccgagagcccccggtgggagaagcgggccggtggctgcgccgcgtgcgttctcactctgaggaagtgcgtggggagccgctgactccggatagcacacccttccgaggggactccccgattcctgggctgggggcctgccgcctggccccacgtctgacgtacggggcgcgagggccactgctccctggacttctgtcggaaccggacgcagtgggaggggtcgcagg

SEQ ID NO: 8 - DNA, 206 bp, homo sapiens
atctgtaaaaatgttgacttctgcttttcagactacgcgcacagcctctttatttcctactgcggcttcattccctcacggaacactgacgccatcgcgaaggaagcatttcgagcacgactgacgctccccttattatttgctaagccgctgcgctcgggtctggctacgatttgctttcagaataacgggaaggtgcaacaaga

SEQ ID NO: 9 - DNA, 27 bp, artificial sequence
  Primer
gaaggaagtatttcgagtacgattgac

SEQ ID NO: 10 - DNA, 19 bp, artificial sequence
  Primer
cccgaacgcaacgacttaa

SEQ ID NO: 11 - DNA, 17 bp, artificial sequence
  Primer
cggaagtcgcgttcgtc

SEQ ID NO: 12 - DNA, 20 bp, artificial sequence
  Primer
gcgtacaactcgtccgctaa

SEQ ID NO: 13 - DNA, 28 bp, artificial sequence
  Probe
ttcgatttcgggattttttgtcgtagtc

SEQ ID NO: 14 - DNA, 20 bp, artificial sequence
  Primer
tgggtgttttggacggtttc

SEQ ID NO: 15 - DNA, 15 bp, artificial sequence
  Primer
cgcctaccctccgcg

SEQ ID NO: 16 - DNA, 26 bp, artificial sequence
  Probe
tcgtttagtttgtggcgatttcgtcg

SEQ ID NO: 17 - DNA, 29 bp, artificial sequence
  Primer
gtttttttgttgatgtaattcgttaggtc

SEQ ID NO: 18 - DNA, 20 bp, artificial sequence
  Primer
caatacccgaaacgacgacg

SEQ ID NO: 19 - DNA, 21 bp, artificial sequence
  Probe
ttcgtcgcgagagggtcggtt

SEQ ID NO: 20 - DNA, 24 bp, artificial sequence
  Primer
gacgacgtatttttttcgtgtttc

SEQ ID NO: 21 - DNA, 16 bp, artificial sequence
  Primer
gcgcacctctcgaccg

SEQ ID NO: 22 - DNA, 25 bp, artificial sequence
  Primer
taagagtaataatggatggatgatg

SEQ ID NO: 23 - DNA, 17 bp, artificial sequence
  Primer
cctcccatctcccttcc

SEQ ID NO: 24 - DNA, 25 bp, artificial sequence
  Probe
atggatgaagaaagaaaggatgagt

SEQ ID NO: 25 - DNA, 24 bp, artificial sequence
  Primer
gtgatggaggaggtttagtaagtt

SEQ ID NO: 26 - DNA, 25 bp, artificial sequence
  Primer
ccaataaaacctactcctcccttaa

SEQ ID NO: 27 - DNA, 30 bp, artificial sequence
  Probe
accaccacccaacacacaataacaaacaca

SEQ ID NO: 28 - DNA, 102 bp, homo sapiens
  misc_feature: bisulphite treated DNA
tagtgttcgaggcggcggcgagtatacgtggcgggttggattgtagatcggttttttcgcggcggagattcgcgatttagcggattgtattagtaggaagat

SEQ ID NO: 29 - DNA, 102 bp, homo sapiens
gtcacgggctccgccgccgctcatgtgcaccgcccgacctaacgtctggccgggagagcgccgcctctgagcgctggatcgcctaacgtagtcgtccttctg

SEQ ID NO: 30 - DNA, 102 bp, homo sapiens
  misc_feature: bisulphite treated DNA
gtttttttgttgatgtaattcgttaggtcgcgagttttcgtcgcgagagggtcggtttgtaatttagttcgttacgtgtattcgtcgtcgtttcgggtattg

SEQ ID NO: 31 - DNA, 26 bp, artificial sequence
  Primer
tttttgttgatgtaattcgttaggtc

SEQ ID NO: 32 - DNA, 20 bp, artificial sequence
  Primer
attacaaaccgaccctctcg

SEQ ID NO: 33 - DNA, 87 bp, homo sapiens
actgccccaggtcttgctgcagccgggaccgcgctctgcagccgcagacccggtccacacggccaggggctacgacccttgggatct

SEQ ID NO: 34 - DNA, 19 bp, artificial sequence
  Primer
agatcccaagggtcgtagc

SEQ ID NO: 35 - DNA, 18 bp, artificial sequence
  Primer
actgccccaggtcttgct

SEQ ID NO: 36 - DNA, 95 bp, homo sapiens
  misc_feature: bisulphite treated DNA
gacgacgtatttttttcgtgtttcgttttgcgtttttttgcgcgtttcgttttttgtatcggagtagcgattcgggaggcggtcgagaggtgcgt

SEQ ID NO: 37 - DNA, 95 bp, homo sapiens
gcgcacctctcggccgcctcccggatcgctgctccggtacagggagcggggcgcgcagaagggcgcagagcgggacacggagagggtgcgtcgtc

SEQ ID NO: 38 - DNA, 95 bp, homo sapiens
  misc_feature: bisulphite treated DNA
gcgtatttttcggtcgtttttcggatcgttgtttcggtatagggagcggggcgcgtagaagggcgtagagcgggatacggagagggtgcgtcgtt

SEQ ID NO: 39 - DNA, 26 bp, artificial sequence
  Primer
tttgtatcggagtagcgattcgggag

SEQ ID NO: 40 - DNA, 92 bp, homo sapiens
agagcgggacacggagagggtgcgtcgtcccgtccccgccccgtcgccgagtcccccggctcgcgcggcgcgcgtctcagccgcaactccgg

SEQ ID NO: 41 - DNA, 17 bp, artificial sequence
  Primer
ggagttgcggctgagac

SEQ ID NO: 42 - DNA, 17 bp, artificial sequence
  Primer
agagcgggacacggaga

SEQ ID NO: 43 - DNA, 110 bp, homo sapiens
  misc_feature: bisulphite treated DNA
cgtttgtttttcgcgtttttgcgacggggtcgttataagttggacgggatgagttaatcggattgtcggggttttaggagtggttgaggcggggtcgtttaaggtattta

SEQ ID NO: 44 - DNA, 110 bp, homo sapiens
tgggtgccttggacggccccgcctcagccactcctggggccccgacagtccggttagctcatcccgtccagcttgtggcgaccccgtcgcaggagcgcggagggcaggcg

SEQ ID NO: 45 - DNA, 110 bp, homo sapiens
  misc_feature: bisulphite treated DNA
tgggtgttttggacggtttcgttttagttatttttggggtttcgatagttcggttagtttatttcgtttagtttgtggcgatttcgtcgtaggagcgcggagggtaggcg

SEQ ID NO: 46 - DNA, 17 bp, artificial sequence
  Primer
gtttttgcgacggggtc

SEQ ID NO: 47 - DNA, 18 bp, artificial sequence
  Primer
taaaaccccgacaatccg

SEQ ID NO: 48 - DNA, 18 bp, artificial sequence
  Primer
taaaaccccgacaatccg

SEQ ID NO: 49 - DNA, 299 bp, homo sapiens
  misc_feature: bisulphite treated DNA
taggaagttgtagtagaaggaggaggcggcggttatttcggatttcgtcgttcggattttcgattcggaagtcgcgttcgtcgtttcggtttcgatttcgggattttttgtcgtagtcgttatttttgggtttttagcggacgagttgtacgcggcgttggaggattattattttgtcgagttgtatcgcgcgttcgtcgtgttcgggggtattttgtttcgtcgaaaggtgcgtttttcgttcgtttttaggatttgtttagttttttttcgattttttatagggtttgttgatttcg

SEQ ID NO: 50 - DNA, 298 bp, homo sapiens
cggagtcagcaggccctgtagggagtcggagaggggctgagcagatcctgaaggcgggcgggggacgcacctttcggcggggcagggtgcccccggacacggcgagcgcgcggtacagctcggcagggtgatagtcctccagcgccgcgtacagctcgtccgctgggggcccaggggtggcggctgcggcagggggtcccggggtcgggaccggagcggcgggcgcgactccgagtcgggagtccgggcggcggggtccggggtggccgccgcctcctccttctgctgcagcttcctg

SEQ ID NO: 51 - DNA, 298 bp, homo sapiens
  misc_feature: bisulphite treated DNA
cggagttagtaggttttgtagggagtcggagaggggttgagtagattttgaaggcgggcgggggacgtatttttcggcggggtagggtgttttcggatacggcgagcgcgcggtatagttcggtagggtgatagttttttagcgtcgcgtatagttcgttcgttgggggtttaggggtggcggttgcggtagggggtttcggggtcgggatcggagcggcgggcgcgatttcgagtcgggagttcgggcggcggggttcggggtggtcgtcgttttttttttttgttgtagttttttg

SEQ ID NO: 52 - DNA, 20 bp, artificial sequence
  Primer
cggattttcgattcggaagt

SEQ ID NO: 53 - DNA, 20 bp, artificial sequence
  Primer
ggtagggtgttttcggatac

SEQ ID NO: 54 - DNA, 21 bp, artificial sequence
  Primer
aacgaacgaactatacgcgac

SEQ ID NO: 55 - DNA, 258 bp, homo sapiens
  misc_feature: bisulphite treated DNA
gatagagatagttttaggtaagttgaaggttcgagagttttcggtgggagaagcgggtcggtggttgcgtcgcgtgcgtttttattttgaggaagtgcgtggggagtcgttgatttcggatagtatattttttcgaggggatttttcgatttttgggttgggggtttgtcgtttggttttacgtttgacgtacggggcgcgagggttattgttttttggatttttgtcggaatcggacgtagtgggaggggtcgtagg

SEQ ID NO: 56 - DNA, 258 bp, homo sapiens
cctgcgacccctcccactgcgtccggttccgacagaagtccagggagcagtggccctcgcgccccgtacgtcagacgtggggccaggcggcaggcccccagcccaggaatcggggagtcccctcggaagggtgtgctatccggagtcagcggctccccacgcacttcctcagagtgagaacgcacgcggcgcagccaccggcccgcttctcccaccgggggctctcggaccttcaacttgcctggggctgtctctgtc

SEQ ID NO: 57 - DNA, 258 bp, homo sapiens
  misc_feature: bisulphite treated DNA
tttgcgattttttttattgcgttcggtttcgatagaagtttagggagtagtggttttcgcgtttcgtacgttagacgtggggttaggcggtaggtttttagtttaggaatcggggagttttttcggaagggtgtgttattcggagttagcggttttttacgtatttttttagagtgagaacgtacgcggcgtagttatcggttcgttttttttatcgggggttttcggatttttaatttgtttggggttgtttttgtt

SEQ ID NO: 58 - DNA, 258 bp, homo sapiens; identical to SEQ ID NO: 7

SEQ ID NO: 59 - DNA, 258 bp, homo sapiens; identical to SEQ ID NO: 56

SEQ ID NO: 60 - DNA, 21 bp, artificial sequence
  Primer
cggagttagcggttttttacg

SEQ ID NO: 61 - DNA, 20 bp, artificial sequence
  Primer
cgataaaaaaaacgaaccga

SEQ ID NO: 62 - DNA, 20 bp, artificial sequence
  Primer
agagtgagaacgtacgcggc

SEQ ID NO: 63 - DNA, 20 bp, artificial sequence
  Primer
caagttgaaggtccgagagc

SEQ ID NO: 64 - DNA, 20 bp, artificial sequence
  Primer
cgcacttcctcagagtgaga

SEQ ID NO: 65 - DNA, 206 bp, homo sapiens
  misc_feature: bisulphite treated DNA
atttgtaaaaatgttgatttttgttttttagattacgcgtatagtttttttattttttattgcggttttatttttttacggaatattgacgttatcgcgaaggaagtatttcgagtacgattgacgttttttttattatttgttaagtcgttgcgttcgggtttggttacgatttgtttttagaataacgggaaggtgtaataaga

SEQ ID NO: 66 - DNA, 28 bp, artificial sequence
  Primer
gcctctaaaaaaacgatcttattacacc

SEQ ID NO: 67 - DNA, 206 bp, homo sapiens
tcttgttgcaccttcccgttattctgaaagcaaatcgtagccagacccgagcgcagcggcttagcaaataataaggggagcgtcagtcgtgctcgaaatgcttccttcgcgatggcgtcagtgttccgtgagggaatgaagccgcagtaggaaataaagaggctgtgcgcgtagtctgaaaagcagaagtcaacatttttacagat

SEQ ID NO: 68 - DNA, 206 bp, homo sapiens
  misc_feature: bisulphite treated DNA
ttttgttgtattttttcgttattttgaaagtaaatcgtagttagattcgagcgtagcggtttagtaaataataaggggagcgttagtcgtgttcgaaatgtttttttcgcgatggcgttagtgtttcgtgagggaatgaagtcgtagtaggaaataaagaggttgtgcgcgtagtttgaaaagtagaagttaatatttttatagat

SEQ ID NO: 69 - DNA, 285 bp, homo sapiens
cacggtcggagggctggtgggctttccttggccgtcgggcccgccacggcgcgggtcttggctgcggggcggaggtggggcgggagagccgaggataagagtttgaggcttttcgaggcgcgtgccgcggcgtccgcctctgcgggactctgcgccgggcgccctcggccggcgcgcccggctcccgctttgtcgccgagggaagcacgcgcgacgcccctcccgtcgccgccgtggcttctttcggtgttcgtgatttgctgagaggctggaaagcagcacggc

SEQ ID NO: 70 - DNA, 285 bp, homo sapiens
  misc_feature: bisulphite treated DNA
tacggtcggagggttggtgggttttttttggtcgtcgggttcgttacggcgcgggttttggttgcggggcggaggtggggcgggagagtcgaggataagagtttgaggtttttcgaggcgcgtgtcgcggcgttcgtttttgcgggattttgcgtcgggcgttttcggtcggcgcgttcggttttcgttttgtcgtcgagggaagtacgcgcgacgtttttttcgtcgtcgtcgtggtttttttcggtgttcgtgatttgttgagaggttggaaagtagtacggt

SEQ ID NO: 71 - DNA, 18 bp, artificial sequence
  Primer
gaaacactaacgccatcg

SEQ ID NO: 72 - DNA, 21 bp, artificial sequence
  Primer
cgtagttagattcgagcgtag

SEQ ID NO: 73 - DNA, 25 bp, artificial sequence
  Primer
aggggagcgttagtcgtgttcgaaa

SEQ ID NO: 74 - DNA, 20 bp, artificial sequence
  Primer
gtttttttcggcgataaagc

SEQ ID NO: 75 - DNA, 20 bp, artificial sequence
  Primer
cgcctctacgaaactctacg

SEQ ID NO: 76 - DNA, 18 bp, artificial sequence
  Primer
cgtcggtcgagggcgttc